European Patent Application EP 4 276 175 A1, published November 15, 2023. Title: Attenuated virus of a flavivirus virus and the use thereof. Applicant: BEIJING SHUNLEI BIOTECHNOLOGY CO., LTD. The sequence listing filed with the application follows.

SEQUENCE LISTING (6 sequences)

SEQ ID NO: 1 - DNA, 10642 bp, West Nile virus
agtagttcgcctgtgtgagctgacaaacttagtagtgtttgtgaggattaacaacaattaacacagtgcgagctgtttcttagcacgaagatctcgatgtctaagaaaccaggagggcccggcaagagccgggctgtcaatatgctaaaacgcggaatgccccgcgtgttgtccttgattggactgaagagggctatgttgagcctgatcgacggcaaggggccaatacgatttgtgttggctctcttggcgttcttcaggttcacagcaattgctccgacccgagcagtgctggatcgatggagaggtgtgaacaaacaaacagcgatgaaacaccttctgagttttaagaaggaactagggaccttgaccagtgctatcaatcggcggagctcaaaacaaaagaaaagaggaggaaagaccggaattgcagtcatgattggcctgatcgccagcgtaggagcagttaccctctctaacttccaagggaaggtgatgatgacggtaaatgctactgacgtcacagatgtcatcacgattccaacagctgctggaaagaacctatgcattgtcagagcaatggatgtgggatacatgtgcgatgatactatcacttatgaatgcccagtgctgtcggctggtaatgatccagaagacatcgactgttggtgcacaaagtcagcagtctacgtcaggtatggaagatgcaccaagacacgccactcaagacgcagtcggaggtcactgacagtgcagacacacggagaaagcactctagcgaacaagaagggggcttggatggacagcaccaaggccacaaggtatttggtaaaaacagaatcatggatcttgaggaaccctggatatgccctggtggcagccgtcattggttggatgcttgggagcaacaccatgcagagagttgtgtttgtcgtgctattgcttttggtggccccagcttacagcttcaactgccttggaatgagcaacagagacttcttggaaggagtgtctggagcaacatgggtggatttggttctcgaaggcgacagctgcgtgactatcatgtctaaggacaagcctaccatcgatgtgaagatgatgaatatggaggcggccaacctggcagaggtccgcagttattgctatttggctaccgtcagcgatctctccaccaaagctgcgtgcccgaccatgggagaagctcacaatgacaaacgtgctgacccagcttttgtgtgcagacaaggagtggtggacaggggctggggcaacggctgcggactatttggcaaaggaagcattgacacatgcgccaaatttgcctgctctaccaaggcaataggaagaaccatcttgaaagagaatatcaagtacgaagtggccatttttgtccatggaccaactactgtggagtcgcacggaaactactccacacaggttggagccactcaggcagggagattcagcatcactcctgcggcgccttcatacacactaaagcttggagaatatggagaggtgacagtggactgtgaaccacggtcagggattgacaccaatgcatactacgtgatgactgttggaacaaagacgttcttggtccatcgtgagtggttcatggacctcaacctcccttggagcagtgctggaagtactgtgtggaggaacagagagacgttaatggagtttgaggaaccacacgccacgaagcagtctgtgatagcattgggctcacaagagggagctctgcatcaagctttggctggagccattcctgtggaattttcaagcaacactgtcaagttgacgtcgggtcatttgaagtgtagagtgaagatggaaaaattgcagttgaagggaacaacctatggcgtctgttcaaaggctttcaagtttcttgggactcccgcagacacaggtcacggcactgtggtgttggaattgcagtacactggcacggatggaccttgtaaagttcctatctcgtcagtggcttcattgaacgacctaacgccagtgggcagattggtcactgtcaacccttttgtttcagtggccacggccaacgctaaggtcctgattgaattggaaccaccctttggagactcatacatagtggtgggcagaggagaacaacagatcaatcaccattggcacaagtctggaagcagcattggcaaagcctttacaaccaccctcaaaggagcgcagagactagccgctctaggagacacagcttgggactttggatcagttggaggggtgttcacctcagttgggaaggctgtccatcaagtgttcggaggagcattccgcttactgttcggaggcatgtcctggataacgcaaggattgctgggggctctcctgttgtggatgggcatcaatgctcgtgataggtccatagctctcacgtttctcgcagttggaggagttctgctcttcctctccgtgaacgtgcacgctgacactgggtgtgccatagacatcagccggcaagagctgagatgtggaagtggagtgttcatacacaatgatgtggaggcttggatggaccgatacaagtattaccctgaaacgccacaaggcctagccaagatcattcagaaagctcataaggaaggagtgtgcggtctacgatcagtttccagactggagcatcaaatgtgggaagcagtgaaggacgagctgaacactcttttgaaggagaatggtgtggaccttagtgtcgtggttgagaaacaggagggaatgtacaagtcagcacctaaacgcctcaccgccaccacggaaaaattggaaattggctggaaggcctggggaaagagtattttatttgcaccagaactcgccaacaacacctttgtggttgatggtccggagaccaaggaatgtccgactcagaatcgcgcttggaatagcttagaagtggaggattttggatttggtctcaccagcactcggatgttcctgaaggtcagagagagcaacacaactgaatgtgactcgaagatcattggaacggctgtcaagaacaacttggcgatccacagtgacctgtcctattggattgaaagcaggctcaatgatacgtggaagcttgaaagggcagttctgggtgaagtcaaatcatgtacgtggcctgagacgcataccttgtggggcgatggaatccttgagagtgacttgataataccagtcacactggcgggaccacgaagcaatcacaatcggagacctgggtacaagacacaaaaccagggcccatgggacgaaggccgggtagagattgacttcgattactgcccaggaactacggtcaccctgagtgagagctgcggacaccgtggacctgccactcgcaccaccacagagagcggaaagttgataacagattggtgctgcaggagctgcaccttaccaccactgcgctaccaaactgacagcggctgttggtatggtatggagatcagaccacagagacatgatgaaaagaccctcgtgcagtcacaagtgaatgcttataatgctgatatgattgacccttttcagttgggccttctggtcgtgttcttggccacccaggaggtccttcgcaagaggtggacagccaagatcagcatgccagctatactgattgctctgctagtcctggtgtttgggggcattacttacactgatgtgttacgctatgtcatcttggtgggggcagctttcgcagaatctaattcgggaggagacgtggtacacttggcgctcatggcgaccttcaagatacaaccagtgtttatggtggcatcgtttctcaaagcgagatggaccaaccaggagaacatcttgttgatgttggcggctgttttctttcaaatggcttatcacgatgcccgccaaattctgctctgggagatccctgatgtgttgaattcactggcggtagcttggatgatactgagagccataacattcacaacgacatcaaacgtggttgttccgctgctagccctgctaacacccgggctgagatgcttgaatctggatgtgtacaggatactgctgttgatggtcggaataggcagcttgatcagggagaagaggagtgcagctgcaaaaaagaaaggagcaagtctgctatgcttggctctagcctcaacaggacttttcaaccccatgatccttgctgctggactgattacatgtgatcccaaccgtaaacgcggatggcccgcaactgaagtgatgacagctgtcggcctgatgtttgccatcgtcggagggctggcagagcttgacattgactccatggccattccaatgactatcgcggggctcatgtttgctgctttcgtgatttctgggaaatcaacagatatgtggattgagagaacggcggacatttcctgggaaagtgatgcagaaattacaggctcgagcgaaagagttgatgtgcggcttgatgatgatggaaacttccagctcatgaatgatccaggagcaccttggaagatatggatgctcagaatggtctgtctcgcgattagtgcgtacaccccctgggcaatcttgccctcagtagttggattttggataactctccaatacacaaagagaggaggcgtgttgtgggacactccctcaccaaaggagtacaaaaagggggacacgaccaccggcgtctacaggatcatgactcgtgggctgctcggcagttatcaagcaggagcgggcgtgatggttgaaggtgttttccacaccctttggcatacaacaaaaggagccgctttgatgagcggagagggccgcctggacccatactggggcagtgtcaaggaggatcgactttgttacggaggaccctggaaattgcagcacaagtggaacgggcaggatgaggtgcagatgattgtggtggaacctggcaagaacgttaagaacgtccagacgaaaccaggggtgttcaaaacacctgaaggagaaatcggggccgtgactttggacttccccactggaacatcaggctcaccaatagtggacaaaaacggtgatgtgattgggctttatggcaatggagtcataatgcccaacggctcatacataagcgcgatagtgcagggtgaaaggatggatgagccaatcccagccggattcgaacctgagatgctgaggaaaaaacagatcactgtactggatctccatcccggcgccggtaaaacaaggaggattctgccacagatcatcaaagaggccataaacagaagactgagaacagccgtgctagcaccaaccagggttgtggctgctgagatggctgaagcactgagaggactgcccatccggtaccagacatccgcagtgcccagagaacataatggaaatgagattgttgatgtcatgtgtcatgctaccctcacccacaggctgatgtctcctcacagggtgccgaactacaacctgttcgtgatggatgaggctcatttcaccgacccagctagcattgcagcaagaggttacatttccacaaaggtcgagctaggggaggcggcggcaatattcatgacagccaccccaccaggcacttcagatccattcccagagtccaattcaccaatttccgacttacagactgagatcccggatcgagcttggaactctggatacgaatggatcacagaatacaccgggaagacggtttggtttgtgcctagtgtcaagatggggaatgagattgccctttgcctacaacgtgctggaaagaaagtagtccaattgaacagaaagtcgtacgagacggagtacccaaaatgtaagaacgatgattgggactttgttatcacaacagacatatctgaaatgggggctaactttaaggcgagcagggtgattgacagccggaagagtgtgaaaccaaccatcataacagaaggagaagggagagtgatcctgggagaaccatctgcagtgacagcagctagtgccgcccagagacgtggacgtatcggtagaaatccgtcgcaagttggtgatgagtactgttatggggggcacacgaatgaagacgactcgaacttcgcccattggactgaggcacgaatcatgctggacaacatcaacatgccaaacggactgatcgctcaattctaccaaccagagcgtgagaaggtatataccatggatggggaataccggctcagaggagaagagagaaaaaactttctggaactgttgaggactgcagatctgccagtttggctggcttacaaggttgcagcggctggagtgtcataccacgaccggaggtggtgctttgatggtcctaggacaaacacaattttagaagacaacaacgaagtggaagtcatcacgaagcttggtgaaaggaagattctgaggccgcgctggattgacgccagggtgtactcggatcaccaggcactaaaggcgttcaaggacttcgcctcgggaaaacgttctcagatagggctcattgaggttctgggaaagatgcctgagcacttcatggggaagacatgggaagcacttgacaccatgtacgttgtggccactgcagagaaaggaggaagagctcacagaatggccctggaggaactgccagatgctcttcagacaattgccttgattgccttattgagtgtgatgaccatgggagtattcttcctcctcatgcagcggaagggcattggaaagataggtttgggaggcgctgtcttgggagtcgcgacctttttctgttggatggctgaagttccaggaacgaagatcgccggaatgttgctgctctcccttctcttgatgattgtgctaattcctgagccagagaagcaacgttcgcagacagacaaccagctagccgtgttcctgatttgtgtcatgacccttgtgagcgcagtggcagccaacgagatgggttggctagataagaccaagagtgacataagcagtttgtttgggcaaagaattgaggtcaaggagaatttcagcatgggagagtttcttttggacttgaggccggcaacagcctggtcactgtacgctgtgacaacagcggtcctcactccactgctaaagcatttgatcacgtcagattacatcaacacctcattgacctcaataaacgttcaggcaagtgcactattcacactcgcgcgaggcttccccttcgtcgatgttggagtgtcggctctcctgctagcagccggatgctggggacaagtcaccctcaccgttacggtaacagcggcaacactccttttttgccactatgcctacatggttcccggttggcaagctgaggcaatgcgctcagcccagcggcggacagcggccggaatcatgaagaacgctgtagtggatggcatcgtggccacggacgtcccagaattagagcgcaccacacccatcatgcagaagaaagttggacagatcatgctgatcttggtgtctctagctgcagtagtagtgaacccgtctgtgaagacagtacgagaagccggaattttgatcacggccgcagcggtgacgctttgggagaatggagcaagctctgtttggaacgcaacaactgccatcggactctgccacatcatgcgtgggggttggttgtcatgtctatccataacatggacactcataaagaacatggaaaaaccaggactaaaaagaggtggggcaaaaggacgcaccttgggagaggtttggaaagaaagactcaaccagatgacaaaagaagagttcactaggtaccgcaaagaggccatcatcgaagtcgatcgctcagcagcaaaacacgccaggaaagaaggcaatgccactggagggcatccagtctctaggggcacagcaaaactgagatggctggtcgaacggaggtttctcgaaccggtcggaaaagtgattgaccttggatgtggaagaggcggttggtgttactatatggcaacccaaaaaagagtccaagaagtcagagggtacacaaagggcggtcccggacatgaagagccccaactagtgcaaagttatggatggaacattgtcaccatgaagagtggagtggatgtgttctacagaccttctgagtgttgtgacaccctcctttgtgacatcggagagtcctcgtcaagtgctgaggttgaagagcataggacgattcgggtccttgaaatggttgaggactggctgcaccgagggccaagggaattttgcgtgaaggtgctctgcccctacatgccgaaagtcatagagaagatggagctgctccaacgccggtatggggggggactggtcagaaacccactctcacggaattccacgcacgagatgtattgggtgagtcgagcttcaggcaatgtggtacattcagtgaatatgaccagccaggtgctcctaggaagaatggaaaaaaggacctggaagggaccccaatacgaggaagatgtaaacttgggaagtggaaccagggcggtgggaaaacccctgctcaactcagacaccagtaaaatcaagaacaggattgaacgactcaggcgtgagtacagttcgacgtggcaccacgatgagaaccacccatatagaacctggaactatcacggcagttatgatgtgaagcccacaggctccgccagttcgctggtcaatggagtggtcaggctcctctcaaaaccatgggacaccatcacgaatgttaccaccatggccatgactgacactactcccttcgggcagcagcgagtgttcaaagagaaggtggacacgaaagctcctgaaccgccagaaggagtgaagtacgtgctcaacgagaccaccaactggttgtgggcgtttttggccagagaaaaacgtccaaggatgtgctctcgagaggagttcataagaaaggtcaacagcaatgcagctttgggtgccatgtttgaagagcagaatcaatggaggagcgccagagaggcagttgaagatccaaaattttgggagatggtggatgaggagcgcgaggcacatctgcggggggaatgtcacacttgcatttacaacatgatgggaaagagagagaaaaaacccggagagttcggaaaggccaagggaagcagagccatttggttcatgtggcttggagctcgctttctggagttcgaggctctgggttttctcaatgaagaccactggcttggaagaaagaactcaggaggaggtgtcgagggcttgggcctccaaaaactgggttacatcctgcgtgaagttggcacccggcctgggggcaagatctatgctgatgacacagctggctgggacacccgcatcacgagagctgacttggaaaatgaagctaaggtgcttgagctgcttgatggggaacatcggcgtcttgccagggccatcattgagctcacctatcgtcacaaagttgtgaaagtgatgcgcccggctgctgatggaagaaccgtcatggatgttatctccagagaagatcagagggggagtggacaagttgtcacctacgccctaaacactttcaccaacctggccgtccagctggtgaggatgatggaaggggaaggagtgattggcccagatgatgtggagaaactcacaaaagggaaaggacccaaagtcaggacctggctgtttgagaatggggaagaaagactcagccgcatggctgtcagtggagatgactgtgtggtaaagcccctggacgatcgctttgccacctcgctccacttcctcaatgctatgtcaaaggttcgcaaagacatccaagagtggaaaccgtcaactggatggtatgattggcagcaggttccattttgctcaaaccatttcactgaattgatcatgaaagatggaagaacactggtggttccatgccgaggacaggatgaattggtaggcagagctcgcatatctccaggggccggatggaacgtccgcgacactgcttgtctggctaagtcttatgcccagatgtggctgcttctgtacttccacagaagagacctgcggctcatggccaacgccatttgctccgctgtccctgtgaattgggtccctaccggaagaaccacgtggtccatccatgcaggaggagagtggatgacaacagaggacatgttggaggtctggaaccgtgtttggatagaggagaatgaatggatggaagacaaaaccccagtggagaaatggagtgacgtcccatattcaggaaaacgagaggacatctggtgtggcagcctgattggcacaagagcccgagccacgtgggcagaaaacatccaggtggctatcaaccaagtcagagcaatcatcggagatgagaagtatgtggattacatgagttcactaaagagatatgaagacacaactttggttgaggacacagtactgtagatatttaaaaaaaaaaaaaaaaaaaaaaaaaaaaaaaaaaaaaaaaaaaaaaaaaaaaaaaaaaaaaaaaaaaaaaaaaaaaaaaaaaaaaaaaaaaaaaaaaaaaaaaaaaaaaaaaaaaaaaaaaaaaaaaaaacagcatattgacacctgggatagactaggagatcttctgctctgcacaaccagccacacggcacagtgcgccgacaatggtggctggtggtgcgagaacacaggatct

SEQ ID NO: 2 - DNA, 10663 bp, Japanese encephalitis virus
agaagtttatctgtgtgaacttcttggcttagtatcgttgagaagaatcgagagattagtgcagtttaaacagttttttagaacggaagataaccatgactaaaaaaccaggagggcccggtaaaaaccgggctatcaatatgctgaaacgcggcctaccccgcgtattcccactagtgggagtgaagagggtagtaatgagcttgttggacggcagagggccagtacgtttcgtgctggctcttatcacgttcttcaagtttacagcattagccccgaccaaggcgcttttaggccgatggaaagcagtggaaaagagtgtggcaatgaaacatcttactagtttcaaacgagaacttggaacactcattgacgccgtgaacaagcggggcagaaagcaaaacaaaagaggaggaaatgaaggctcaatcatgtggctcgcgagcttggcagttgtcatagcttgtgcaggagccatgaagttgtcgaatttccaggggaagcttttgatgaccatcaacaacacggacattgcagacgttatcgtgattcccacctcaaaaggagagaacagatgctgggtccgggcaatcgacgtcggctacatgtgtgaggacactatcacgtacgaatgtcctaagcttaccatgggcaatgatccagaggatgtggattgctggtgtgacaaccaagaagtctacgtccaatatggacggtgcacgcggaccaggcattccaagcgaagcaggagatccgtgtcggtccaaacacatggggagagttcactagtgaataaaaaagaggcttggctggattcaacgaaagccacacgatatctcatgaaaactgagaactggatcataaggaatcctggctatgctttcctggcggcggtacttggctggatgcttggcagtaacaacggtcaacgcgtggtatttaccatcctcctgctgttggtcgctccggcttacagttttaattgtctgggaatgggcaatcgcgacttcatagaaggagccagtggagccacttgggtggacttggtgctggaaggagatagctgcttgacaatcatggcaaacgacaaaccaacattggacgtccgcatgattaacatcgaagctagccaacttgctgaggtcagaagttactgctatcatgcttcagtcactgacatctcgacggtggctcggtgccccacgactggagaagcccacaacgagaagcgagctgatagtagctatgtgtgcaaacaaggcttcactgaccgtgggtggggcaacggatgtggacttttcgggaagggaagcattgacacatgtgcaaaattctcctgcaccagtaaagcgattgggagaacaatccagccagaaaacatcaaatacgaagttggcatttttgtgcatggaaccaccacttcggaaaaccatgggaattattcagcgcaagttggggcgtcccaggcggcaaagtttacagtaacacccaatgctccttcgataaccctcaaacttggtgactacggagaagtcacactggactgtgagccaaggagtggactgaacactgaagcgttttacgtcatgaccgtggggtcaaagtcatttctggtccatagggagtggtttcatgacctcgctctcccctggacgtccccttcgagcacagcgtggagaaacagagaactcctcatggaatttgaagaggcgcacgccacaaaacagtccgttgttgctcttgggtcacaggaaggaggcctccatcaggcgttggcaggagccatcgtggtggagtactcaagctcagtgaagttaacatcaggccacctgaaatgtaggctgaaaatggacaaactggctctgaaaggcacaacctatggcatgtgtacagaaaaattctcgttcgcgaaaaatccggcggacactggtcacggaacagttgtcattgaactctcctactctgggagtgatggcccctgcaaaattccgattgtttccgttgcgagcctcaatgacatgacccccgttgggcggctggtgacagtgaaccccttcgtcgcgacttccagtgccaactcaaaggtgctggtcgagatggaaccccccttcggagactcctacatcgtagttggaaggggagacaagcagatcaaccaccattggcacaaagctggaagcacgctgggcaaggccttttcaacaactttgaagggagctcaaagactggcagcgttgggcgacacagcctgggactttggctctattggaggggtcttcaactccataggaaaagccgttcaccaagtgtttggtggtgccttcagaacactctttgggggaatgtcttggatcacacaagggctaatgggtgccctactgctctggatgggcgtcaacgcacgagaccgatcaattgctttggccttcttagccacagggggtgtgctcgtgttcttagcgaccaatgtgcatgctgacactggatgtgccattgacatcacaagaaaagagatgagatgtggaagtggcatcttcgtgcacaacgacgtggaagcctgggtggataggtataaatatttgccagaaacgcccagatccctagcgaagatcgtccacaaagcgcacaaggaaggcgtgtgcggagtcagatctgtcactagactggagcaccaaatgtgggaagccgtaagggacgaattgaacgtcctgctcaaagagaatgcagtggacctcagtgtggttgtgaacaagcccgtgggaagatatcgctcagcccctaaacgcctatccatgacgcaagagaagtttgaaatgggctggaaagcatggggaaaaagcatcctctttgccccggaattggctaactccacatttgtcgtagatggacctgagacaaaggaatgccctgatgagcacagagcttggaacagcatgcaaatcgaagacttcggctttggcatcacatcaacccgtgtgtggctgaaaattagagaggagagcactgacgagtgtgatggagcgatcataggcacggctgtcaaaggacatgtggcagtccatagtgacttgtcgtactggattgagagtcgctacaacgacacatggaaacttgagagggcagtctttggagaggtcaaatcttgcacttggccagagacacacaccctttggggagatgatgttgaggaaagtgaactcatcattccgcacaccatagccggaccaaaaagcaagcacaatcggagggaagggtataagacacaaaaccagggaccttgggatgagaatggcatagtcttggactttgattattgcccagggacaaaagtcaccattacagaggattgtagcaagagaggcccttcggtcagaaccactactgacagtggaaagttgatcactgactggtgctgtcgcagttgctcccttccgcccctacgattccggacagaaaatggctgctggtacggaatggaaatcagacctgttaggcatgatgaaacaacactcgtcagatcacaggttgatgctttcaatggtgaaatggttgacccttttcagctgggccttctggtgatgtttctggccacccaggaggtccttcgcaagaggtggacggccagattgaccattcctgcggttttgggggccctacttgtgctgatgcttgggggcatcacttacactgatttggcgaggtatgtggtgctagtcgctgctgctttcgcagaggccaacagtggaggagacgtcctgcaccttgctttgattgccgtttttaagatccaaccagcatttctagtgatgaacatgcttagcacgagatggacgaaccaagaaaacgtggttctggtcctaggggctgcctttttccaattggcctcagtagatctgcaaataggagtccacggaatcctgaatgccgccgctatagcatggatgattgtccgagcgatcaccttccccacaacctcctccgtcaccatgccagtcttagcgcttctaactccggggatgagggctctatacctagacacttacagaatcatcctcctcgtcatagggatttgctccctgctgcacgagaggaaaaagaccatggcaaaaaagaaaggagctgtactcttgggcttagcgctcacatccactggatggttctcgcccaccactatagctgccggactaatggtctgcaacccaaacaagaagagagggtggccagctactgagtttttgtcggcagttggattgatgtttgccatcgtaggtggtttggccgagttggatattgaatccatgtcaatacccttcatgctggcaggtctcatggcagtgtcctacgtggtgtcaggaaaagcaacagatatgtggcttgaacgggccgccgacatcagctgggagatggatgctgcaatcacaggaagcagtcggaggctggatgtgaaactggatgatgacggagattttcacttgattgatgatcccggtgttccatggaaggtctgggtcctgcgcatgtcttgcattggcttagccgccctcacgccttgggccatcgttcccgccgctttcggttattggctcactttaaaaacaacaaaaagagggggcgtgttttgggacacgccatccccaaaaccttgctcaaaaggagacaccactacaggagtctaccgaattatggctagagggattcttggcacttaccaggccggcgtcggagtcatgtacgagaatgttttccacacactatggcacacaactagaggagcagccattatgagtggagaaggaaaattgacgccatactggggtagtgtgagagaagaccgcatagcttacggaggcccatggaggtttgaccgaaaatggaatggaacagatgacgtgcaagtgatcgtggtagaaccggggaaggctgcagtaaacatccagacaaaaccaggagtgtttcggactcccttcggggaggttggggctgttagtctggattacccgcgaggaacatccggctcacccattctggattccaatggagacattataggcctatacggcaatggagttgagcttggcgatggctcatacgtcagcgccatcgtgcagggtgaccgtcaggaggaaccagtcccagaagcttacaccccaaacatgttgagaaagagacagatgactgtgctagatttgcaccctggttcagggaaaaccaggaaaattctgccacaaataattaaggacgccatccagcagcgcctaagaacagctgtgttggcaccgacgcgggtggtagcagcagaaatggcagaagctttgagagggctcccagtacgatatcaaacttcagcagtgcagagagagcaccaagggaatgaaatagtggatgtgatgtgccacgccactctgacccatagactgatgtcaccgaacagagtgcccaactacaacctatttgtcatggatgaagctcatttcaccgacccagccagtatagccgcacgaggatacattgctaccaaggtggaattaggggaggcagcagccatctttatgacagcgaccccgcctggaaccacggatccttttcctgactcaaatgccccaatccatgatttgcaagatgagataccagacagggcatggagcagtggatacgaatggatcacagaatatgcgggtaaaaccgtgtggtttgtggcgagcgtaaaaatggggaatgagattgcaatgtgcctccaaagagcggggaaaaaggtcatccaactcaaccgcaagtcctatgacacagaatacccaaaatgtaagaatggagactgggattttgtcattaccaccgacatctctgaaatgggggccaacttcggtgcgagcagggtcatcgactgtagaaagagcgtgaaacccaccatcttagaagagggagaaggcagagtcatcctcggaaacccatctcccataaccagtgcaagcgcagctcaacggaggggcagagtaggcagaaaccccaaccaagttggagatgaataccactatgggggggctaccagtgaagatgacagtaacctagcccattggacagaggcaaagatcatgttagacaacatacacatgcccaatggactggtggcccagctctatggaccagagagggaaaaggctttcacaatggatggcgaataccgtctcagaggtgaagaaaagaaaaacttcttagagctgcttaggacggctgacctcccggtgtggctggcctacaaggtggcgtccaatggcattcagtacaccgacagaaagtggtgttttgatgggccgcgtacgaatgccatactggaggacaacaccgaggtagagatagtcacccggatgggtgagaggaaaatcctcaagccgagatggcttgatgcaagagtttatgcagatcaccaagccctcaagtggttcaaagactttgcagcagggaagagatcagccgttagcttcatagaggtgctcggtcgcatgcctgagcatttcatgggaaagacgcgggaagctttagacaccatgtacttggttgcaacggctgagaaaggtgggaaagcacaccgaatggctctcgaagagctgccagatgcactggaaaccatcacacttattgtcgccattactgtgatgacaggaggattcttcctactaatgatgcagcgaaagggtatagggaagatgggtcttggagctctagtgctcacgctagctaccttcttcctgtgggcggcagaggttcctggaaccaaaatagcagggaccctgctgatcgccctgctgctgatggtggttctcatcccagaaccggaaaaacagaggtcacagacagataaccaactggcggtgtttctcatctgtgtcttgaccgtggttggagtggtggcagcaaacgagtacgggatgctagaaaaaaccaaagcagatctcaagagcatgtttggcggaaagacgcaggcatcaggactgactggattgccaagcatggcactggacctgcgtccagccacagcctgggcactgtatggggggagcacagtcgtgctaacccctcttctgaagcacctgatcacgtcggaatacgtcaccacatcgctagcctcaattaactcacaagctggctcattattcgtcttgccacgaggcgtgccttttaccgacctagacttgaccgttggcctcgtcttccttggctgttggggtcaaatcaccctcacaacgtttctgacagccatggttctggcgacacttcactatgggtacatgctccctggatggcaagcagaagcactcagggctgcccagagaaggacagcggctggaataatgaagaatgccgttgttgacggaatggtcgccactgatgtgcctgaactggaaaggactactcctctgatgcaaaagaaagtcggacaggtgctcctcataggggtaagcgtggcagcgttcctcgtcaaccctaatgtcaccactgtgagagaagcaggggtgttggtgacggcggctacgcttactttgtgggacaatggagccagtgccgtttggaattccaccacagccacgggactctgccatgtcatgcgaggtagctacctggctggaggctccattgcttggactctcatcaagaacgctgataagccctccttgaaaaggggaaggcctgggggcaggacgctaggggagcagtggaaggaaaaactaaatgccatgagcagagaagagttttttaaataccggagagaggccataatcgaggtggaccgcactgaagcacgcagggccagacgtgaaaataacatagtgggaggacatccggtttcgcgaggctcagcaaaactccgttggctcgtggagaaaggatttgtctcgccaataggaaaagtcattgatctagggtgtgggcgtggaggatggagctactacgcagcaaccctgaagaaggtccaggaagtcagaggatacacgaaaggtggggcgggacatgaagaaccgatgctcatgcagagctacggctggaacctggtctccctgaagagtggagtggacgtgttttacaaaccttcagagcccagtgacaccctgttctgtgacataggggaatcctccccaagtccagaagtagaagaacaacgcacactacgcgtcctagagatgacatctgactggttgcaccgaggacctagagagttctgcattaaagttctctgcccttacatgcccaaggttatagaaaaaatggaagttctgcagcgccgcttcggaggtgggctagtgcgtctccccctgtcccgaaactccaatcacgagatgtattgggttagtggagccgctggcaatgtggtgcacgctgtgaacatgaccagccaggtactactggggcgaatggatcgcacagtgtggagagggccaaagtatgaggaagatgtcaacctagggagcggaacaagagccgtgggaaagggagaagtccatagcaatcaggagaaaatcaagaagagaatccagaagcttaaagaagaattcgccacaacgtggcacaaagaccctgagcatccataccgcacttggacataccacggaagctatgaagtgaaggctactggctcagccagctctctcgtcaacggagtggtgaagctcatgagcaaaccttgggacgccattgccaacgtcaccaccatggccatgactgacaccaccccttttggacagcaaagagttttcaaggagaaagttgacacgaaggctcctgagccaccagctggagccaaggaagtgctcaacgagaccaccaactggctgtgggcccacttgtcacgggaaaaaagaccccgcttgtgcaccaaggaagaattcataaagaaagtcaacagcaacgcggctcttggagcagtgttcgctgaacagaatcaatggagcacggcgcgtgaggctgtggatgacccgcggttttgggagatggttgatgaagagagggaaaaccatctgcgaggagagtgtcacacatgtatctacaacatgatgggaaaaagagagaagaagcctggagagtttggaaaagctaaaggaagcagggccatttggttcatgtggcttggagcacggtatctagagtttgaagctttggggttcctgaatgaagaccattggctgagccgagagaattcaggaggtggagtggaaggctcaggcgtccaaaagctgggatacatcctccgtgacatagcaggaaagcaaggagggaaaatgtacgctgatgataccgccgggtgggacactagaattaccagaactgatttagaaaatgaagctaaggtactggagctcctagacggtgaacaccgcatgctcgcccgagccataattgaactgacttacaggcacaaagtggtcaaggtcatgagacctgcagcagaaggaaagaccgtgatggacgtgatatcaagagaagatcaaagggggagtggacaggtggtcacttatgctcttaacactttcacgaacatcgctgtccagctcgtcaggctgatggaggctgagggggtcattggaccacaacacttggaacagctacctaggaaaaacaagatagctgtcaggacctggctctttgagaatggagaggagagagtgaccaggatggcgatcagcggagacgactgtgtcgtcaagccgctggacgacagattcgccacagccctccacttcctcaacgcaatgtcaaaggtcagaaaagacatccaggaatggaagccttcgcatggctggcacgattggcagcaagttcccttctgctctaaccattttcaggagattgtgatgaaagatggaaggagtatagttgtcccgtgcagaggacaggatgagctgataggcagggctcgcatctctccaggagctggatggaatgtgaaggacacagcttgcctggccaaagcatatgcacagatgtggctactcctatacttccatcgcagggacttgcgtctcatggcaaatgcgatttgctcagcagtgccagtggattgggtgcccacaggcaggacatcctggtcaatacactcgaaaggagagtggatgaccacggaagacatgctgcaggtctggaacagagtctggattgaagaaaatgaatggatgatggacaagactccaatcacaagctggacagacgttccgtatgtgggaaagcgtgaggacatctggtgtggcagcctcatcggaacgcgatccagagcaacctgggctgagaacatctatgcggcgataaaccaggttagagctgtcattgggaaagaaaattatgttgactacatgacctcactcaggagatacgaagacgtcttgatccaggaagacagggtcatctagtgtgataaaaaaaaaaaaaaaaaaaaaaaaaaaaaaaaaaaaaaaaaaaaaaaaaaaaaaaaaaaaaaaaaaaaaaaaaaaaaaaaaaaaaaaaaaaaaaaaaaaaaaaaaaaaaaaaaaaaaaaaaaaaaaaaaaaaaaaaaaaaaaaaaaaaaaagcatattgacacctgggaatagactgggagatcttctgctctatctcaacatcagctactaggcacagagcgccgaagtatgtagctggtagtgaggaagaacacaggatct

SEQ ID NO: 3 - DNA, 10523 bp, Dengue virus type 2
agttgttagtctacgtggaccgacaaagacagattctttgagggagctaagctcaacgtagttctaacagttttttaattagagagcagatctctgatgaataaccaacgaaaaaaggcgagaaatacgcctttcaatatgctgaaacgcgagagaaaccgcgtgtcgactgtacaacagctgacaaagagattctcacttggaatgctgcagggacgaggaccattaaaactgttcatggccctggtggcgttccttcgtttcctaacaatcccaccaacagcagggatactgaagagatggggaacaattaaaaaatcaaaagccattaatgttttgagagggttcaggaaagagattggaaggatgctgaacatcttgaacaggagacgcagaactgcaggcatgatcattatgctgattccaacagtgatggcgttccatttaaccacacgtaacggagaaccacacatgatcgtcagtagacaagagaaagggaaaagtcttctgtttaaaacagaggatggtgtgaacatgtgtaccctcatggccatggaccttggtgaattgtgtgaagatacaatcacgtacaagtgtccttttctcaggcagaatgaaccagaagacatagattgttggtgcaactctacgtccacatgggtaacttatgggacgtgtaccaccacaggagaacacagaagagaaaaaagatcagtggcactcgttccacatgtgggaatgggactggagacacgaactgaaacatggatgtcatcagaaggggcctggaaacatgcccagagaattgaaacttggatcttgagacatccaggctttaccataatggcagcaatcctggcatacaccataggaacgacacatttccaaagagccctgattttcatcttactgacagctgtcgctccttcaatgacaatgcgttgcataggaatatcaaatagagactttgtagaaggggtttcaggaggaagctgggttgacatagtcttagaacatggaagctgtgtgacgacgatggcaaaaaacaaaccaacattggattttgaactgataaaaacagaagccaaacaacctgccactctaaggaagtactgtatagaggcaaagctgaccaacacaacaacagattctcgctgcccaacacaaggagaacccagcctaaatgaagagcaggacaaaaggttcgtctgcaaacactccatggtggacagaggatggggaaatggatgtggattatttggaaaaggaggcattgtgacctgtgctatgttcacatgcaaaaagaacatgaaaggaaaagtcgtgcaaccagaaaacttggaatacaccattgtgataacacctcactcaggggaagagcatgcagtcggaaatgacacaggaaaacatggcaaggaaatcaaaataacaccacagagttccatcacagaagcagagttgacaggctatggcactgtcacgatggagtgctctccgagaacgggcctcgacttcaatgagatggtgttgctgcaaatggaaaataaagcttggctggtgcacaggcaatggttcctagacctgccgttgccatggctgcccggagcggacacacaaggatcaaattggatacagaaagagacattggtcactttcaaaaatccccatgcgaagaaacaggatgttgttgttttgggatcccaagaaggggccatgcacacagcactcacaggggccacagaaatccagatgtcatcaggaaacttactgttcacaggacatctcaagtgcaggctgaggatggacaaactacagctcaaaggaatgtcatactctatgtgcacaggaaagtttaaagttgtgaaggaaatagcagaaacacaacatggaacaatagttatcagagtacaatatgaaggggacggttctccatgtaagatcccttttgagataatggatttggaaaaaagacatgttttaggtcgcctgattacagtcaacccaatcgtaacagaaaaagatagcccagtcaacatagaagcagaacctccattcggagacagctacatcatcataggagtagagccgggacaattgaagctcaactggtttaagaaaggaagttctatcggccaaatgattgagacaacaatgaggggagcgaagagaatggccattttaggtgacacagcttgggattttggatccctgggaggagtgtttacatctataggaaaggctctccaccaagttttcggagcaatctatggggctgccttcagtggggtctcatggactatgaaaatactcataggagtcattatcacatggataggaatgaattcacgcagcacctcactgtctgtgtcactagtattggtgggagtcgtgacgctgtatttgggagttatggtgcaggccgatagtggttgcgttgtgagctggaaaaacaaagaactgaagtgtggcagtgggattttcatcacagacaacgtgcacacatggacagaacaatacaagttccaaccagaatccccttcaaagctagcttcagctatccagaaagctcatgaagagggcatttgtggaatccgctcagtaacaagactggaaaatctgatgtggaaacaaataacaccagaattgaatcacattctatcagaaaatgaggtgaagttgactattatgacaggagacatcaaaggaatcatgcaggcaggaaaacgatctctgcagccccagcccactgagctgaagtattcatggaaaacatggggcaaagcgaaaatgctctctacagagtctcataaccagacctttctcattgatggccccgaaacagcagaatgccccaacacaaacagagcttggaattcgctggaagttgaagactatggctttggagtattcaccaccaatatatggctaaagttgagagaaaagcaggatgtattctgcgactcaaaactcatgtcagcggccataaaagacaacagagccgtccatgccgatatgggttattggatagaaagtgcactcaatgacacatggaagatagagaaagcctctttcatcgaagttaaaagctgccactggccaaagtcacacaccctctggagtaatggagtgttagaaagtgagatgataattccaaagaatttcgctggaccagtgtcacaacacaactacagaccaggctaccatacacaaacagcaggaccatggcatctaggtaagcttgagatggactttgatttctgcgaaggaaccacagtggtggtgactgaggactgtggaaatagaggaccctctttaagaacaactactgcctctggaaaactcataacagaatggtgctgccgatcttgcacattaccaccgctaagatacagaggtgaggacggatgctggtacgggatggaaatcagaccattgaaagagaaagaagagaatttggtcaactccttggtcacagccggacatgggcagattgacaacttttcactaggagtcttgggaatggcattgttcctggaagaaatgctcaggacccgagtaggaacgaaacatgcaatactactagttgcagtttcttttgtgacattgatcacagggaacatgtcctttagagacctgggaagagtgatggttatggtgggcgctactatgacggatgacataggtatgggcgtgacttatcttgccctactagcagccttcaaagtcagaccaacttttgcagctggactactcttgagaaagttgacctccaaggaattgatgatgactaccataggaatcgtactcctctcccagagcaccataccagagaccattcttgaactgactgatgcgttagccttgggcatgatggtccttaaaatggtgagaaaaatggaaaagtatcaattggcagtgactatcatggctatcttgtgcgtcccaaatgcagtgatattacaaaacgcatggaaagtgagttgcacaatattggcagtggtgtccgtttccccactgttcttaacatcctcacagcagaaagcggattggataccattagcattgacgatcaagggtctcaatccaacagctatttttctaacaaccctttcaagaaccaacaagaaaaggagctggccactaaatgaggctatcatggcagtcgggatggtgagcattttggccagttcactcctaaagaatgacattcccatgacaggaccattagtggctggagggctcctcactgtgtgctacgtgctcactggacgatcggccgatttggaactggagagagccgccgatgtcaaatgggaagatcaggcagagatatcagggagctctccaatcctgtcaataacaatatcagaagatggtagcatgtcgataaaaaacgaagaggaagaacaaacactgaccatactcattagaacaggattgctggtgatctcaggactttttcctgtatcaataccaatcacggcagcagcatggtacctgtgggaagtgaagaaacaacgggctggagtattgtgggatgtcccttcacccccacccgtgggaaaggctgaactggaagatggagcctatagaatcaagcaaaaagggattcttggatattcccagatcggagccggagtttacaaagaaggaacattccatacaatgtggcatgtcacacgcggcgctgttctaatgcataaaggaaagaggattgaaccatcatgggcggacgttaagaaagacctaatatcatatggaggaggctggaagctagaaggagaatggaaggaaggagaagaagtccaggtcttggcattggagcctggaaaaaatccaagagccgtccaaacaaaacctggtcttttcaaaaccaacgccggaaccataggtgccgtatctctggacttttctcctggaacctcaggatctccaatcatcgacaaaaaaggaaaagttgtgggtctttatggtaatggtgttgttacaaggagtggagcatatgtgagtgctatagcccagactgaaaaaagtattgaagacaatccagagatcgaagatgatatttttcgaaagagaaaattgaccatcatggacctccacccaggagcgggaaagacgaagagataccttccggccatagtcagagaggctataaaacggggcctgaggacattaatcctggcccccactagagtcgtggcagctgaaatggaggaagccctaagaggacttccaataagataccaaaccccagccatcagagctgagcacaccgggcgggagattgtggacctaatgtgtcatgccacattcactatgaggctgctatcaccagttagagtgccaaattacaacctgatcatcatggacgaagcccatttcacagacccagcaagtatagcggctagaggatacatctcaactcgagtagagatgggtgaggcagctgggattttcatgacagccactcctccgggaagcagagacccattccctcagagcaatgcaccaatcatggatgaagaaagagaaatccctgaacgttcgtggagttctggacatgagtgggtcacggattttaaagggaagactgtttggttcgttccaagtataaaagcaggaaatgatatagcagcttgcctgagaaaaaatggaaagaaagtgatacaactcagtaggaagacctttgattctgagtatgtcaagactagaaccaatgattgggacttcgtggtcacaactgacatttcagaaatgggtgccaacttcaaggctgagagggttatagaccccagacgctgcatgaaaccagttatactaacagatggtgaagagcgggtgatcctggcaggacctatgccagtgacccactctagtgcagcacaaagaagagggagaataggaagaaatccaaaaaatgaaaatgaccagtacatatacatgggggaacctctggaaaatgatgaagactgtgcacactggaaagaagctaaaatgctcctagataacatcaacacacctgaaggaatcattcctagcatgttcgaaccagagcgtgaaaaggtggatgccattgatggtgaataccgcttgagaggagaagcaaggaaaacctttgtggacctaatgagaagaggagacctaccagtctggttggcctacagagtggcagctgaaggcatcaactacgcagacagaaggtggtgttttgatggaattaagaacaaccaaatcttggaagaaaatgtggaggtggaaatctggacaaaagaaggggaaaggaagaaattaaaacccagatggttggatgccaggatctactctgacccactgacgctaaaggaattcaaggagtttgcagctggaagaaagtccctgaccctgaacctaatcacagaaatgggtaggcttccaactttcatgactcagaaggcaagagacgcactggacaacttagcagtgctgcacacggctgaagcaggtggaagggcgtacaatcatgctctcagtgaactgccggagaccctggagacattgcttttactgacacttctggctacagtcacaggaggaatctttttattcttgatgtccggaaggggtatagggaagatgaccctgggaatgtgctgcataatcacggccagtattctcctatggtacgcacaaatacagccacactggatagcagcttcaataatactggagttttttctcatagttttgcttattccagaaccagaaaagcagagaacaccccaagataaccaattgacctacgttgtcatagccatcctcacagtggtggccgcaaccatggcaaacgagatgggtttcctggaaaaaacgaagaaagatctcggattgggaagcattacaacccagcaacccgagagcaacatcctggacatagatctacgtcccgcatcagcatggacgctgtatgctgtggccacaacatttgtcacaccaatgttgagacacagcattgaaaattcctcagtgaacgtgtccctaacagctattgccaaccaagccacagtgttaatgggtcttgggaaaggatggccattgtcaaagatggacatcggagttccccttctcgccattggatgctactcacaagtcaaccccataactctcacagcagctcttttcttactggtagcacattatgccatcatagggccaggactccaagcaaaagcaaccagggaagctcagaaaagagcagcagcgggcatcatgaaaaacccaactgtcgatggaataacagtgattgacctagatccaataccctatgatccaaagtttgaaaagcagttgggacaagtaatgctcctagtcctctgcgtgactcaagtgttgatgatgaggactacatgggctctgtgtgaggcgttaaccttagcgaccgggcctatctccacattgtgggaaggaaatccagggaggttttggaacactaccattgcagtgtcaatggctaacatttttagagggagttacttggccggagctggacttctcttttccatcatgaagaacacaaccaacacgagaaggggaaccggtaacataggagagacgcttggagagaaatggaaaagccgattgaacgcattggggaaaagtgaattccagatctacaagaaaagtggaatccaggaagtggatagaaccttagcaaaagaaggcattaaaagaggagaaacggaccatcacgctgtgtcgcgaggctcagcaaaactgagatggttcgtcgagagaaatatggtcacaccagaagggaaagtagtggacctcggttgcggcagaggaggctggtcatactattgtgggggactaaagaatgtaagagaagtcaaaggcctgacaaaaggaggaccaggacatgaagaacccatccccatgtcaacatatgggtggaatctagtacgtcttcaaagtggagttgacgttttcttcactccgccagaaaagtgtgacacattgttgtgtgacataggggagtcgtcaccaaatcccacggtagaagcaggacgaacactcagagtccttaacttagtggaaaattggttgaacaacaacacccaattttgcataaaggttctcaacccatacatgccctcagtcatagaaaaaatggaagcactacaaaggaaatatggaggagccttagtgaggaatccactctcacgaaactccacacatgagatgtactgggtatccaatgcctccgggaacatagtgtcatcagtgaacatgatttcaaggatgttgatcaacagattcacaatgagacacaagaaagccacttacgagccagatgtagacctcggaagcggaacccgcaacatcggaattgaaagtgagataccaaacctagacataatcgggaaaagaatagaaaaaataaaacaagagcatgaaacatcatggcactatgaccaagaccacccatacaaaacgtgggcttaccatggcagctatgaaacaaaacaaactggatcagcatcatccatggtgaacggagtggtcagactgctgacaaaaccttgggacgtcgtccccatggtgacacagatggcaatgacagacacgactccatttggacaacagcgcgtttttaaagaaaaagtggacacgagaacccaagaaccgaaagaaggcacaaagaaactaatgaaaatcacggcagagtggctttggaaagaactagggaagaaaaagacacctaggatgtgcactagagaagaattcacaagaaaggtgagaagcaatgcagccttgggggccatattcactgatgagaacaagtggaagtcggcacgtgaggctgttgaagatagtaggttttgggagctggttgacaaggaaaggaatctccatcttgaaggaaagtgtgaaacatgtgtgtataacatgatgggaaaaagagagaagaagctaggggagttcggcaaggcaaaaggcagcagagccatatggtacatgtggcttggagcacgcttcttagagtttgaagccctaggattcttgaatgaagatcactggttctccagagagaactccttgagtggagtggaaggagaagggctgcacaagctaggttacattttaagagacgtgagcaagaaagagggaggagcaatgtatgccgatgacaccgcaggatgggacacaagaatcacactagaagacctaaaaaatgaagaaatggtaacaaaccacatggaaggagaacacaagaaactagccgaggccattttcaaattaacgtaccaaaacaaggtggtgcgtgtgcaaagaccaacaccaagaggcacagtaatggatatcatatcgagaagagaccaaagaggtagtggacaagttggtacctatggactcaatactttcaccaatatggaagcccaactaatcagacagatggagggagaaggagtcttcaaaagcattcagcacctgacagtcacagaagaaatcgccgtgcaaaactggttagcaagagtagggcgcgaaaggttatcaagaatggccatcagtggagatgattgtgttgtgaaacctttagatgacaggttcgcaagcgctttaacagctctaaatgacatgggaaaggttaggaaagacatacaacaatgggaaccttcaagaggatggaacgattggacacaagtgcccttctgttcacaccatttccatgagttaatcatgaaagacggacgcgtacttgtagttccatgcagaaaccaagatgaactgattggtagagcccgaatttcccaaggagctgggtggtctttgcgagagacggcctgtttggggaagtcctacgcccaaatgtggagcttgatgtacttccacagacgtgacctcaggctggcggctaatgctatttgctcggcagtcccatcacattgggttccaacaagtagaacaacctggtccatacacgccaaacatgaatggatgacaacggaagacatgctgacagtctggaacagggtgtggattcaagaaaacccatggatggaagacaaaactccagtggaatcatgggaggaaatcccatacttggggaaaagagaagaccaatggtgcggctcattgattgggctaacaagcagggccacctgggcaaagaacatccaaacagcaataaatcaagttagatcccttataggcaatgaggaatacacagattacatgccatccatgaaaagattcagaagagaagaggaagaggcaggagtcctgtggtagaaggcaaaaaaaaaaaaaaaaaaaaaaaaaaaaaaaaaaaaaaaaaaaaaaaaaaaaaaaaaaaaaaaaaaaaaaaaaaaaaaaaaaaaaaaaaaaaaaaaaaaaaaaaaaaaaaaaaaaaaaaaaaaaaaaaaaaaaaaaaaaacagcatattgacgctgggaaagaccagagatcctgctgtctcctcagcatcattccaggcacagaacgccagaaaatggaatggtgctgttgaatcaacaggttct

SEQ ID NO: 4 - DNA, 10775 bp, Yellow fever virus
agtaaatcctgtgtgctaattgaggtgcattggtctgcaaatcgagttgctaggcaataaacacatttggattaattttaatcgttcgttgagcgattagcagagaactgaccagaacatgtctggtcgtaaagctcagggaaaaaccctgggcgtcaatatggtacgacgaggagttcgctccttgtcaaacaaaataaaacaaaaaacaaaacaaattggaaacagacctggaccttcaagaggtgttcaaggatttatctttttctttttgttcaacattttgactggaaaaaagatcacagcccacctaaagaggttgtggaaaatgctggacccaagacaaggcttggctgttctaaggaaagtcaagagagtggtggccagtttgatgagaggattgtcctcaaggaaacgccgttcccatgatgttctgactgtgcaattcctaattttgggaatgctgttgatgacgggtggagtgaccttggtgcggaaaaacagatggttgctcctaaatgtgacatctgaggacctcgggaaaacattctctgtgggcacaggcaactgcacaacaaacattttggaagccaagtactggtgcccagactcaatggaatacaactgtcccaatctcagtccaagagaggagccagatgacattgattgctggtgctatggggtggaaaacgttagagtcgcatatggtaagtgtgactcagcaggcaggtctaggaggtcaagaagggccattgacttgcctacgcatgaaaaccatggtttgaagacccggcaagaaaaatggatgactggaagaatgggtgaaaggcaactccaaaagattgagagatggttcgtgaggaaccccttttttgcagtgacggctctgaccattgcctaccttgtgggaagcaacatgacgcaacgagtcgtgattgccctactggtcttggctgttggtccggcctactcagctcactgcattggaattactgacagggatttcattgagggggtgcatggaggaacttgggtttcagctaccctggagcaagacaagtgtgtcactgttatggcccctgacaagccttcattggacatctcactagagacagtagccattgatagacctgctgaggtgaggaaagtgtgttacaatgcagttctcactcatgtgaagattaatgacaagtgccccagcactggagaggcccacctagctgaagagaacgaaggggacaatgcgtgcaagcgcacttattctgatagaggctggggcaatggctgtggcctatttgggaaagggagcattgtggcatgcgccaaattcacttgtgccaaatccatgagtttgtttgaggttgatcagaccaaaattcagtatgtcatcagagcacaattgcatgtaggggccaagcaggaaaattggaataccgacattaagactctcaagtttgatgccctgtcaggctcccaggaagtcgagttcattgggtatggaaaagctacactggaatgccaggtgcaaactgcggtggactttggtaacagttacatcgctgagatggaaacagagagctggatagtggacagacagtgggcccaggacttgaccctgccatggcagagtggaagtggcggggtgtggagagagatgcatcatcttgtcgaatttgaacctccgcatgccgccactatcagagtactggccctgggaaaccaggaaggctccttgaaaacagctcttactggcgcaatgagggttacaaaggacacaaatgacaacaacctttacaaactacatggtggacatgtttcttgcagagtgaaattgtcagctttgacactcaaggggacatcctacaaaatatgcactgacaaaatgttttttgtcaagaacccaactgacactggccatggcactgttgtgatgcaggtgaaagtgtcaaaaggagccccctgcaggattccagtgatagtagctgatgatcttacagcggcaatcaataaaggcattttggttacagttaaccccatcgcctcaaccaatgatgatgaagtgctgattgaggtgaacccaccttttggagacagctacattatcgttgggagaggagattcacgtctcacttaccagtggcacaaagagggaagctcaataggaaagttgttcactcagaccatgaaaggcgtggaacgcctggccgtcatgggagacaccgcctgggatttcagctccgctggagggttcttcacttcggttgggaaaggaattcatacggtgtttggctctgcctttcaggggctatttggcggcttgaactggataacaaaggtcatcatgggggcggtacttatatgggttggcatcaacacaagaaacatgacaatgtccatgagcatgatcttggtaggagtgatcatgatgtttttgtctctaggagttggggcggatcaaggatgcgccatcaactttggcaagagagagctcaagtgcggagatggtatcttcatatttagagactctgatgactggctgaacaagtactcatactatccagaagatcctgtgaagcttgcatcaatagtgaaagcctcttttgaagaagggaagtgtggcctaaattcagttgactcccttgagcatgagatgtggagaagcagggcagatgagatcaatgccatttttgaggaaaacgaggtggacatttctgttgtcgtgcaggatccaaagaatgtttaccagagaggaactcatccattttccagaattcgggatggtctgcagtatggttggaagacttggggtaagaaccttgtgttctccccagggaggaagaatggaagcttcatcatagatggaaagtccaggaaagaatgcccgttttcaaaccgggtctggaattctttccagatagaggagtttgggacgggagtgttcaccacacgcgtgtacatggacgcagtctttgaatacaccatagactgcgatggatctatcttgggtgcagcggtgaacggaaaaaagagtgcccatggctctccaacattttggatgggaagtcatgaagtaaatgggacatggatgatccacaccttggaggcattagattacaaggagtgtgagtggccactgacacatacgattggaacatcagttgaagagagtgaaatgttcatgccgagatcaatcggaggcccagttagctctcacaatcatatccctggatacaaggttcagacgaacggaccttggatgcaggtaccactagaagtgaagagagaagcttgcccagggactagcgtgatcattgatggcaactgtgatggacggggaaaatcaaccagatccaccacggatagcgggaaagttattcctgaatggtgttgccgctcctgcacaatgccgcctgtgagcttccatggtagtgatgggtgttggtatcccatggaaattaggccaaggaaaacgcatgaaagccatctggtgcgctcctgggttacagctggagaaatacatgctgtcccttttggtttggtgagcatgatgatagcaatggaagtggtcctaaggaaaagacagggaccaaagcaaatgttggttggaggagtagtgctcttgggagcaatgctggtcgggcaagtaactctccttgatttgctgaaactcacagtggctgtgggattgcatttccatgagatgaacaatggaggagacgccatgtatatggcgttgattgctgccttttcaatcagaccagggctgctcatcggctttgggctcaggaccctatggagccctcgggaacgccttgtgctgaccctaggagcagccatggtggagattgccttgggtggcgtgatgggcggcctgtggaagtatctaaatgcagtttctctctgcatcctgacaataaatgctgttgcttctaggaaagcatcaaataccatcttgcccctcatggctctgttgacacctgtcactatggctgaggtgagacttgccgcaatgttcttttgtgccgtggttatcataggggtccttcaccagaatttcaaggacacctccatgcagaagactatacctctggtggccctcacactcacatcttacctgggcttgacacaaccttttttgggcctgtgtgcatttctggcaacccgcatatttgggcgaaggagtatcccagtgaatgaggcactcgcagcagctggtctagtgggagtgctggcaggactggcttttcaggagatggagaacttccttggtccgattgcagttggaggactcctgatgatgctggttagcgtggctgggagggtggatgggctagagctcaagaagcttggtgaagtttcatgggaagaggaggcggagatcagcgggagttccgcccgctatgatgtggcactcagtgaacaaggggagttcaagctgctttctgaagagaaagtgccatgggaccaggttgtgatgacctcgctggccttggttggggctgccctccatccatttgctcttctgctggtccttgctgggtggctgtttcatgtcaggggagctaggagaagtggggatgtcttgtgggatattcccactcctaagatcatcgaggaatgtgaacatctggaggatgggatttatggcatattccagtcaaccttcttgggggcctcccagcgaggagtgggagtggcacagggaggggtgttccacacaatgtggcatgtcacaagaggagctttccttgtcaggaatggcaagaagttgattccatcttgggcttcagtaaaggaagaccttgtcgcctatggtggctcatggaagttggaaggcagatgggatggagaggaagaggtccagttgatcgcggctgttccaggaaagaacgtggtcaacgtccagacaaaaccgagcttgttcaaagtgaggaatgggggagaaatcggggctgtcgctcttgactatccgagtggcacttcaggatctcctattgttaacaggaacggagaggtgattgggctgtacggcaatggcatccttgtcggtgacaactccttcgtgtccgccatatcccagactgaggtgaaggaagaaggaaaggaggagctccaagagatcccgacaatgctaaagaaaggaatgacaactgtccttgattttcatcctggagctgggaagacaagacgtttcctcccacagatcttggccgagtgcgcacggagacgcttgcgcactcttgtgttggcccccaccagggttgttctttctgaaatgaaggaggcttttcacggcctggacgtgaaattccacacacaggctttttccgctcacggcagcgggagagaagtcattgatgccatgtgccatgccaccctaacttacaggatgttggaaccaactagggttgttaactgggaagtgatcattatggatgaagcccattttttggatccagctagcatagccgctagaggttgggcagcgcacagagctagggcaaatgaaagtgcaacaatcttgatgacagccacaccgcctgggactagtgatgaatttccacattcaaatggtgaaatagaagatgttcaaacggacatacccagtgagccctggaacacagggcatgactggatcctagctgacaaaaggcccacggcatggttccttccatccatcagagctgcaaatgtcatggctgcctctttgcgtaaggctggaaagagtgtggtggtcctgaacaggaaaacctttgagagagaataccccacgataaagcagaagaaacctgactttatattggccactgacatagctgaaatgggagccaacctttgcgtggagcgagtgctggattgcaggacggcttttaagcctgtgcttgtggatgaagggaggaaggtggcaataaaagggccacttcgtatctccgcatcctctgctgctcaaaggagggggcgcattgggagaaatcccaacagagatggagactcatactactattctgagcctacaagtgaaaataatgcccaccacgtctgctggttggaggcctcaatgctcttggacaacatggaggtgaggggtggaatggtcgccccactctatggcgttgaaggaactaaaacaccagtttcccctggtgaaatgagactgagggatgaccagaggaaagtcttcagagaactagtgaggaattgtgacctgcccgtttggctttcgtggcaagtggccaaggctggtttgaagacgaatgatcgtaagtggtgttttgaaggccctgaggaacatgagatcttgaatgacagcggtgaaacagtgaagtgcagggctcctggaggagcaaagaagcctctgcgcccaaggtggtgtgatgaaagggtgtcatctgaccagagtgcgctgtctgaatttattaagtttgctgaaggtaggaggggagctgctgaagtgctagttgtgctgagtgaactccctgatttcctggctaaaaaaggtggagaggcaatggataccatcagtgtgttcctccactctgaggaaggctctagggcttaccgcaatgcactatcaatgatgcctgaggcaatgacaatagtcatgctgtttatactggctggactactgacatcgggaatggtcatctttttcatgtctcccaaaggcatcagtagaatgtctatggcgatgggcacaatggccggctgtggatatctcatgttccttggaggcgtcaaacccactcacatctcctatgtcatgctcatattctttgtcctgatggtggttgtgatccccgagccagggcaacaaaggtccatccaagacaaccaagtggcatacctcattattggcatcctgacgctggtttcagcggtggcagccaacgagctaggcatgctggagaaaaccaaagaggacctctttgggaagaagaacttaattccatctagtgcttcaccctggagttggccggatcttgacctgaagccaggagctgcctggacagtgtacgttggcattgttacaatgctctctccaatgttgcaccactggatcaaagtcgaatatggcaacctgtctctgtctggaatagcccagtcagcctcagtcctttctttcatggacaaggggataccattcatgaagatgaatatctcggtcataatgctgctggtcagtggctggaattcaataacagtgatgcctctgctctgtggcatagggtgcgccatgctccactggtctctcattttacctggaatcaaagcgcagcagtcaaagcttgcacagagaagggtgttccatggcgttgccaagaaccctgtggttgatgggaatccaacagttgacattgaggaagctcctgaaatgcctgccctttatgagaagaaactggctctatatctccttcttgctctcagcctagcttctgttgccatgtgcagaacgcccttttcattggctgaaggcattgtcctagcatcagctgccttagggccgctcatagagggaaacaccagccttctttggaatggacccatggctgtctccatgacaggagtcatgagggggaatcactatgcttttgtgggagtcatgtacaatctatggaagatgaaaactggacgccgggggagcgcgaatggaaaaactttgggtgaagtctggaagagggaactgaatctgttggacaagcgacagtttgagttgtataaaaggaccgacattgtggaggtggatcgtgatacggcacgcaggcatttggccgaagggaaggtggacaccggggtggcggtctccagggggaccgcaaagttaaggtggttccatgagcgtggctatgtcaagctggaaggtagggtgattgacctggggtgtggccgcggaggctggtgttactacgctgctgcgcaaaaggaagtgagtggggtcaaaggatttactcttggaagagacggccatgagaaacccatgaatgtgcaaagtctgggatggaacatcatcaccttcaaggacaaaactgatatccaccgcctagaaccagtgaaatgtgacacccttttgtgtgacattggagagtcatcatcgtcatcggtcacagagggggaaaggaccgtgagagttcttgatactgtagaaaaatggctggcttgtggggttgacaacttctgtgtgaaggtgttagctccatacatgccagatgttctcgagaaactggaattgctccaaaggaggtttggcggaacagtgatcaggaaccctctctccaggaattccactcatgaaatgtactacgtgtctggagcccgcagcaatgtcacatttactgtgaaccaaacatcccgcctcctgatgaggagaatgaggcgtccaactggaaaagtgaccctggaggctgacgtcatcctcccaattgggacacgcagtgttgagacagacaagggacccctggacaaagaggccatagaagaaagggttgagaggataaaatctgagtacatgacctcttggttttatgacaatgacaacccctacaggacctggcactactgtggctcctatgtcacaaaaacctcaggaagtgcggcgagcatggtaaatggtgttattaaaattctgacatatccatgggacaggatagaggaggtcacaagaatggcaatgactgacacaaccccttttggacagcaaagagtgtttaaagaaaaagttgacaccagagcaaaggatccaccagcgggaactaggaagatcatgaaagttgtcaacaggtggctgttccgccacctggccagagaaaagaaccccagactgtgcacaaaggaagaatttattgcaaaagtccgaagtcatgcagccattggagcttacctggaagaacaagaacagtggaagactgccaatgaggctgtccaagacccaaagttctgggaactggtggatgaagaaaggaagctgcaccaacaaggcaggtgtcggacttgtgtgtacaacatgatggggaaaagagagaagaagctgtcagagtttgggaaagcaaagggaagccgtgccatatggtatatgtggctgggagcgcggtatcttgagtttgaggccctgggattcctgaatgaggaccattgggcttccagggaaaactcaggaggaggagtggaaggcattggcttacaatacctaggatatgtgatcagagacctggctgcaatggatggtggtggattctacgcggatgacaccgctggatgggacacgcgcatcacagaggcagaccttgatgatgaacaggagatcttgaactacatgagcccacatcacaaaaaactggcacaagcagtgatggaaatgacatacaagaacaaagtggtgaaagtgttgagaccagccccaggagggaaagcctacatggatgtcataagtcgacgagaccagagaggatccgggcaggtagtgacttatgctctgaacaccatcaccaacttgaaagtccaattgatcagaatggcagaagcagagatggtgatacatcaccaacatgttcaagattgtgatgaatcagttctgaccaggctggaggcatggctcactgagcacggatgtgacagactgaagaggatggcggtgagtggagacgactgtgtggtccggcccatcgatgacaggttcggcctggccctgtcccatctcaacgccatgtccaaggttagaaaggacatatctgaatggcagccatcaaaagggtggaatgattgggagaatgtgcccttctgttcccaccacttccatgaactacagctgaaggatggcaggaggattgtggtgccttgccgagaacaggacgagctcattgggagaggaagggtgtctccaggaaacggctggatgatcaaggaaacagcttgcctcagcaaagcctatgccaacatgtggtcactgatgtattttcacaaaagggacatgaggctactgtcattggctgtttcctcagctgttcccacctcatgggttccacaaggacgcacaacatggtcgattcatgggaaaggggagtggatgaccacggaagacatgcttgaggtgtggaacagagtatggataaccaacaacccacacatgcaggacaagacaatggtgaaaaaatggagagatgtcccttatctaaccaagagacaagacaagctgtgcggatcactgattggaatgaccaatagggccacctgggcctcccacatccatttagtcatccatcgtatccgaacgctgattggacaggagaaatacactgactacctaacagtcatggacaggtattctgtggatgctgacctgcaactgggtgagcttatctgaaacaccatctaacaggaataaccgggatacaaaccacgggtggagaaccggactccccacaacctgaaaccgggatataaaccacggctggagaaccggactccgcacttaaaatgaaacagaaaccgggataaaaactacggatggagaaccggactccacacattgagacagaagaaaaaaaaaaaaaaaaaaaaaaaaaaaaaaaaaaaaaaaaaaaaaaaaaaaaaaaaaaaaaaaaaaaaaaaaaaaaaaaaaaaaaaaaaaaaaaaaaaaaaaaaaaaaaaaaaaaaaaaaaaaaaaaaaaaaccatattgacgccagggaaagaccggagtggttctctgcttttcctccagaggtctgtgagcacagtttgctcaagaataagcagacctttggatgacaaacacaaaaccac

SEQ ID NO: 5 - DNA, 10625 bp, zika virus
agttgttgatctgtgtgagtcagactgcgacagttcgagtttgaagcgaaagctagcaacagtatcaacaggttttattttggatttggaaacgagagtttctggtcatgaaaaacccaaaaaagaaatccggaggattccggattgtcaatatgctaaaacgcggagtagcccgtgtgagcccctttgggggcttgaagaggctgccagccggacttctgctgggtcatgggcccatcaggatggtcttggcgattctagccttcttgagattcacggcaatcaagccatcactgggtctcatcaatagatggggttcagtggggaaaaaagaggctatggaaataataaagaagttcaagaaagatctggctgccatgctgagaataatcaatgctaggaaggagaagaagagacgaggcgcagatactaatgtcggaattgttggcctcctgctgaccacagctatggcagcggaggtcactagacgtgggagtgcatactatatgtacttggacagaaacgatgctggggaggccatatcttttccaaccacattggggatgaataagtgttatatacagatcatggatcttggacacatgtgtgatgccaccatgagctatgaatgccctatgctggatgagggggtggaaccagatgacgtcgattgttggtgcaacacgacgtcaacttgggttgtgtacggaacctgccatcacaaaaaaggtgaagcacggagatctagaagagctgtgacgctcccctcccattccactaggaagctgcaaacgcggtcgcaaacttggttggaatcaagagaatacacaaagcacttgattagagtcgaaaattggatattcaggaaccctggcttcgcgttagcagcagctgccatcgcttggcttttgggaagctcaacgagccaaaaagtcatatacttggtcatgatactgctgattgccccggcatacagcatcaggtgcataggagtcagcaatagggactttgtggaaggtatgtcaggtgggacttgggttgatgttgtcttggaacatggaggttgtgtcaccgtaatggcacaggacaaaccgactgtcgacatagagctggttacaacaacagtcagcaacatggcggaggtaagatcctactgctatgaggcatcaatatcggacatggcttcggacagccgctgcccaacacaaggtgaagcctaccttgacaagcaatcagacactcaatatgtctgcaaaagaacgttagtggacagaggctggggaaatggatgtggactttttggcaaagggagcctggtgacatgcgctaagtttgcatgctccaagaaaatgaccgggaagagcatccagccagagaatctggagtaccggataatgctgtcagttcatggctcccagcacagtgggatgatcgttaatgacacaggacatgaaactgatgagaatagagcgaaggttgagataacgcccaattcaccaagagccgaagccaccctggggggttttggaagcctaggacttgattgtgaaccgaggacaggccttgacttttcagatttgtattacttgactatgaataacaagcactggttggttcacaaggagtggttccacgacattccattaccttggcacgctggggcagacaccggaactccacactggaacaacaaagaagcactggtagagttcaaggacgcacatgccaaaaggcaaactgtcgtggttctagggagtcaagaaggagcagttcacacggcccttgctggagctctggaggctgagatggatggtgcaaagggaaggctgtcctctggccacttgaaatgtcgcctgaaaatggataaacttagattgaagggcgtgtcatactccttgtgtaccgcagcgttcacattcaccaagatcccggctgaaacactgcacgggacagtcacagtggaggtacagtacgcagggacagatggaccttgcaaggttccagctcagatggcggtggacatgcaaactctgaccccagttgggaggctgataaccgctaaccccgtaatcactgaaagcactgagaactccaagatgatgctggaacttgatccaccatttggggactcttacattgtcataggagtcggggagaagaagatcacccaccactggcacaggagtggcagcaccattggaaaagcatttgaagccactgtgagaggtgccaggagaatggcagtcttgggagacacagcctgggactttggatcagttggaggcgctctcaactcattgggcaagggcatccatcaaatttttggagcagctttcaaatcattgtttggaggaatgtcctggttctcacaaattctcattggaacgttgctgatgtggttgggtctgaacacaaagaatggatctatttcccttatgtgcttggccttagggggagtgttgatcttcttatccacagccgtctctgctgatgtggggtgctcggtggacttctcaaagaaggagacgagatgcggtacaggggtgttcgtctataacgacgttgaagcctggagggacaggtacaagtaccatcctgactccccccgtagattggcagcagcagtcaagcaagcctgggaagatggtatctgtgggatctcctctgtttcaagaatggaaaacatcatgtggagatcagtagaaggggagctcaacgcaatcctggaagagaatggagttcaactgacggtcgttgtgggatctgtaaaaaaccccatgtggagaggtccacagagattgcccgtgcctgtgaacgagctgccccacggctggaaggcttgggggaaatcgtacttcgtcagagcagcaaagacaaataacagctttgtcgtggatggtgacacactgaaggaatgcccactcaaacatagagcatggaacagctttcttgtggaggatcatgggttcggggtatttcacactagtgtctggctcaaggttagagaagattattcattagagtgtgatccagccgttattggaacagctgttaagggaaaggaggctgtacacagtgatctaggctactggattgagagtgagaagaatgacacatggaggctgaagagggcccatctgatcgagataaaaacatgtgaatggccaaagtcccacacattgtggacagatggaatagaagagagtgatctgatcatacccaagtctttagctgggccactcagccatcacaataccagagagggctacaggacccaaatgaaagggccatggcacagtgaagagcttgaaattcggtttgaggaatgcccaggcaccaaggtccacgtggaggaaacatgtggaacaagaggaccatctctgagatcaaccactgcaagcggaagggtgatcgaggaatggtgctgcagggagtgcacaatgcccccactgtcgttccaggctaaagatggctgttggtatggaatggagataaggcccaggaaagaaccagaaagtaacttagtaaggtcaatggtgactgcaggatcaactgatcacatggatcacttctcccttggagtgcttgtgattctgctcatggtgcaggaagggctgaagaagagaatgaccacaaagatcatcataagcacatcaatggcagtgctggtagctatgatcctgggaggattttcaatgagtgacctggctaagcttgcaattttgatgggtgccaccttcgcggaaatgaacactggaggagatgtagctcatctggcgctgatagcggcattcaaagtcagaccagcgttgctggtatctttcatcttcagagctaattggacaccccgtgaaagcatgctgctggccttggcctcgtgtcttttgcaaactgcgatctccgccttggaaggcgacctgatggttctcatcaatggttttgctttggcctggttggcaatacgagcgatggttgttccacgcactgataacatcaccttggcaatcctggctgctctgacaccactggcccggggcacactgcttgtggcgtggagagcaggccttgctacttgcggggggtttatgctcctctctctgaagggaaaaggcagtgtgaagaagaacttaccatttgtcatggccctgggactaaccgctgtgaggctggtcgaccccatcaacgtggtgggactgctgttgctcacaaggagtgggaagcggagctggccccctagcgaagtactcacagctgttggcctgatatgcgcattggctggagggttcgccaaggcagatatagagatggctgggcccattgccgcggtcggtctgctaattgtcagttacgtggtctcaggaaagagtgtggacatgtacattgaaagagcaggtgacatcacatgggaaaaagatgcggaagtcactggaaacagtccccggcttgatgtggcgctagatgagagtggtgatttctccctggtggaggatgacggtccccccatgagagagatcatactcaaggtggtcctgatgaccatctgtggcatgaacccaatagccataccctttgcagctggagcgtggtacgtatacgtgaagactggaaaaaggagtggagctctatgggatgtgcctgctcccaaggaagtaaaaaagggggagaccacagatggagtgtacagagtgatgactcgtagactgctaggttcaacacaagttggagtgggagttatgcaagagggggtctttcacaccatgtggcacgtcacaaaaggatccgcgctgagaagcggtgaagggagacttgatccatactggggagatgtcaagcaggatctggtgtcatactgtggtccatggaagctagatgccgcctgggacgggcacagcgaggtgcagctcttggccgtgccccccggagagagagcgaggaacatccagactctgcccggaatatttaagacaaaggatggggacattggagcggttgcgctggattacccagcaggaacttcaggatctccaatcctagacaagtgtgggagagtgataggactttatggcaatggggtcgtgatcaaaaatgggagttatgttagtgccatcacccaagggaggagggaggaagagactcctgttgagtgcttcgagccttcgatgctgaagaagaagcagctaactgtcttagacttgcatcctggagctgggaaaaccaggagagttcttcctgaaatagtccgtgaagccataaaaacaagactccgtactgtgatcttagctccaaccagggttgtcgctgccgaaatggaggaagcccttagagggcttccagtgcgttatatgacaacagcagtcaatgtcacccactctggaacagaaatcgtcgacttaatgtgccatgccaccttcacttcacgtctactacagccaatcagagtccccaactataatctgtatattatggatgaggcccacttcacagatccctcaagtatagcagcaagaggatacatttcaacaagggttgagatgggcgaggcggctgccatcttcatgaccgccacgccaccaggaacccgtgacgcatttccggactccaactcaccaattatggacaccgaagtggaagtcccagagagagcctggagctcaggctttgattgggtgacggatcattctggaaaaacagtctggtttgttccaagcgtgaggaacggcaatgagatcgcagcttgtctgacaaaggctggaaaacgggtcatacagctcagcagaaagacttttgagacagagttccagaaaacaaaacatcaagagtgggactttgtcgtgacaactgacatttcagagatgggcgccaactttaaagctgaccgtgtcatagattccaggagatgcctaaagccggtcatacttgatggcgagagagtcattctggctggacccatgcctgtcacacatgccagcgctgcccagaggagggggcgcataggcaggaatcccaacaaacctggagatgagtatctgtatggaggtgggtgcgcagagactgacgaagaccatgcacactggcttgaagcaagaatgctccttgacaatatttacctccaagatggcctcatagcctcgctctatcgacctgaggccgacaaagtagcagccattgagggagagttcaagcttaggacggagcaaaggaagacctttgtggaactcatgaaaagaggagatcttcctgtttggctggcctatcaggttgcatctgccggaataacctacacagatagaagatggtgctttgatggcacgaccaacaacaccataatggaagacagtgtgccggcagaggtgtggaccagacacggagagaaaagagtgctcaaaccgaggtggatggacgccagagtttgttcagatcacgcggccctgaagtcattcaaggagtttgccgctgggaaaagaggagcggcttttggagtgatggaagccttgggaacactgccaggacacatgacagagagattccaggaagccattgacaacctcgctgtgctcatgcgggcagagactggaagcaggccttacaaagccgcggcggcccaattgccggagaccctagagaccattatgcttttggggttgctgggaacagtctcgctgggaatctttttcgtcttgatgaggaacaagggcatagggaagatgggctttggaatggtgactcttggggccagcgcatggctcatgtggctctcggaaattgagccagccagaattgcatgtgtcctcattgttgtgttcctattgctggtggtgctcatacctgagccagaaaagcaaagatctccccaggacaaccaaatggcaatcatcatcatggtagcagtaggtcttctgggcttgattaccgccaatgaactcggatggttggagagaacaaagagtgacctaagccatctaatgggaaggagagaggagggggcaaccataggattctcaatggacattgacctgcggccagcctcagcttgggccatctacgctgccttgacaactttcattaccccagccgtccaacatgcagtgaccacttcatacaacaactactccttaatggcgatggccacgcaagctggagtgttgtttggtatgggcaaagggatgccattctacgcatgggactttggagtcccgctgctaatgataggttgctactcacaattaacacccctgaccctaatagtagccatcattttgctcgtggcgcactacatgtacttgatcccagggctgcaggcagcagctgcgcgtgctgcccagaagagaacggcagctggcatcatgaagaaccctgttgtggatggaatagtggtgactgacattgacacaatgacaattgacccccaagtggagaaaaagatgggacaggtgctactcatagcagtagccgtctccagcgccatactgtcgcggaccgcctgggggtggggggaggctggggccctgatcacagctgcaacttccactttgtgggaaggctctccgaacaagtactggaactcctctacagccacttcactgtgtaacatttttaggggaagttacttggctggagcttctctaatctacacagtaacaagaaacgctggcttggtcaagagacgtgggggtggaacaggagagaccctgggagagaaatggaaggcccgcttgaaccagatgtcggccctggagttctactcctacaaaaagtcaggcatcaccgaggtgtgcagagaagaggcccgccgcgccctcaaggacggtgtggcaacgggaggccatgctgtgtcccgaggaagtgcaaagctgagatggttggtggagcggggatacctgcagccctatggaaaggtcattgatcttggatgtggcagagggggctggagttactacgccgccaccatccgcaaagttcaagaagtgaaaggatacacaaaaggaggccctggtcatgaagaacccatgttggtgcaaagctatgggtggaacatagtccgtcttaagagtggggtggacgtctttcatatggcggctgagccgtgtgacacgttgctgtgtgacataggtgagtcatcatctagtcctgaagtggaagaagcacggacgctcagagtcctttccatggtgggggattggcttgaaaaaagaccaggagccttttgtataaaagtgttgtgcccatacaccagcactatgatggaaaccctggagcgactgcagcgtaggtatgggggaggactggtcagagtgccactctcccgcaactctacacatgagatgtactgggtctctggagcgaaaagcaacaccataaaaagtgtgtccaccacgagccagctcctcttggggcgcatggacgggcccaggaggccagtgaaatatgaggaggatgtgaatctcggctctggcacgcgggctgtggtaagctgcgctgaagctcccaacatgaagatcattggtaaccgcattgaaaggatccgcagtgagcacgcggaaacgtggttctttgacgagaaccacccatataggacatgggcttaccatggaagctatgaggcccccacacaagggtcagcgtcctctctaataaacggggttgtcaggctcctgtcaaaaccctgggatgtggtgactggagtcacaggaatagccatgaccgacaccacaccgtatggtcagcaaagagttttcaaggaaaaagtggacactagggtgccagatccccaagaaggcactcgtcaggttatgagcatggtctcttcctggttgtggaaagagctaggcaaacacaaacggccacgagtctgtaccaaagaagagttcatcaacaaggttcgtagcaatgcagcattaggggcaatatttgaagaggaaaaagagtggaagactgcagtggaagctgtgaacgatccaaggttctgggctctagtggacaaggaaagagagcaccacctgagaggagagtgccagagttgtgtgtacaacatgatgggaaaaagagaaaagaaacaaggggaatttggaaaggccaagggcagccgcgccatctggtatatgtggctaggggctagatttctagagttcgaagcccttggattcttgaacgaggatcactggatggggagagagaactcaggaggtggtgttgaagggctgggattacaaagactcggatatgtcctagaagagatgagtcgcataccaggaggaaggatgtatgcagatgacactgctggctgggacacccgcatcagcaggtttgatctggagaatgaagctctaatcaccaaccaaatggagaaagggcacagggccttggcattggccataatcaagtacacataccaaaacaaagtggtaaaggtccttagaccagctgaaaaagggaagacagttatggacattatttcgagacaagaccaaagggggagcggacaagttgtcacttacgctcttaacacatttaccaacctagtggtgcaactcattcggagtatggaggctgaggaagttctagagatgcaagacttgtggctgctgcggaggtcagagaaagtgaccaactggctgcagagcaacggatgggataggctcaaacgaatggcagtcagtggagatgattgcgttgtgaggccaattgatgataggtttgcacatgccctcaggttcttgaatgatatggggaaagttaggaaggacacacaagagtggaaaccctcaactggatgggacaactgggaggaagttccgttttgctcccaccacttcaacaagctccatctcaaggacgggaggtccattgtggttccctgccgccaccaagatgaactgattggccgggcccgcgtctctccaggggcgggatggagcatccgggagactgcttgcctagcaaaatcatatgcgcaaatgtggcagctcctttatttccacagaagggacctccgactgatggccaatgccatttgttcatctgtgccagttgactgggttccaactgggagaactacctggtcaatccatggaaagggagaatggatgaccactgaagacatgcttgtggtgtggaacagagtgtggattgaggagaacgaccacatggaagacaagaccccagttacgaaatggacagacattccctatttgggaaaaagggaagacttgtggtgtggatctctcatagggcacagaccgcgcaccacctgggctgagaacattaaaaacacagtcaacatggtgcgcaggatcataggtgatgaagaaaagtacatggactacctatccacccaagttcgctacttgggtgaagaagggtctacacctggagtgctgtaagcaccaaaaaaaaaaaaaaaaaaaaaaaaaaaaaaaaaaaaaaaaaaaaaaaaaaaaaaaaaaaaaaaaaaaaaaaaaaaaaaaaaaaaaaaaaaaaaaaaaaaaaaaaaaaaaaaaaaaaaaaaaaaaaaaaaacagcatattgacgctgggaaagaccagagactccatgagtttccaccacgctggccgccaggcacagatcgccgaatagcggcggccggtgtggggaaatccatggtttct

SEQ ID NO: 6 - DNA, 10903 bp, Tick-borne encephalitis virus
agattttcttgcacgtgcatgcgtttgcttcggacagcattagcagcggttggtttgaaagagatattcttttgtttctaccagtcgtgaacgtgttgagaaaaagacagcttaggagaacaagagctggggatggtcaagaaggccatcctgaaaggtaaggggggcggtccccctcgacgagtgtcgaaagagaccgcaacgaagacgcgtcaacccagagtccaaatgccaaatgggcttgtgttgatgcgcatgatggggatcttgtggcatgccgtagccggcaccgcgagaaaccccgtattgaaggcgttctggaactcagtccctctgaaacaggcaacagcagcactgcggaagatcaaaaggacggtgagtgccctaatggttggcttgcaaaaacgtgggaaaaggaggtcagcgacggactggatgagctggttgctggtcatcactctgttggggatgacgcttgctgcaacggtgaggaaagaaagggatggctcaactgtgatcagagctgaaggaaaggatgcagcaactcaggtgcgtgtggagaatggcacctgtgtgatcctggctactgacatggggtcatggtgtgatgattcactgtcctatgagtgtgtgaccatagatcaaggagaagagcctgttgacgtggattgtttttgccggaacgttgatggagtctatctggagtacggacgctgtgggaaacaggaaggctcacggacaaggcgctcagtgctgatcccatcccatgctcagggagagctgacgggaaggggacacaaatggctagaaggagactcgctgcgaacacaccttactagagttgagggatgggtctggaagaacaagctacttgccttggcaatggttaccgttgtgtggttgaccctggagagtgtggtgaccagggttgccgttcttgttgtgctcctgtgtttggcaccggtttacgcttcgcgttgcacacacttggaaaacagggactttgtgactggtactcaggggactacgagggtcaccttggtgctggaactgggtggatgtgttactataacagctgaggggaagccttcaatggatgtgtggcttgacgccatttaccaggagaaccctgctaagacacgtgagtactgtttacacgccaagttgtcggacactaaggttgcagccagatgcccaacaatgggaccagccactttggctgaagaacaccagggtggcacagtgtgtaagagagatcagagtgatcgaggctggggcaaccactgtggactgtttggaaagggtagcattgtggcctgtgtcaaggcggcttgtgaggcaaaaaagaaagccacaggacatgtgtacgacgccaacaaaatagtgtacacggtcaaagtcgaaccacacacgggagactatgttgccgcaaacgagacacatagtgggaggaagacggcatccttcacaatttcttcagagaaaaccattttgactatgggtgagtatggagatgtgtctttgttgtgcagggtcgctagtggcgttgacttggcccagaccgtcatccttgagcttgacaagacagtggaacaccttccaacggcttggcaggtccatagggactggttcaatgatctggctctgccatggaaacatgagggagcgcaaaactggaacaacgcagaaagactggttgaatttggggctcctcacgctgtcaagatggacgtgtacaacctcggagaccagactggagtgttactgaaggctctcgctggggttcctgtggcacacattgagggaaccaagtaccacctgaagagtggccacgtgacctgcgaagtgggactggaaaaactgaagatgaaaggtcttacgtacacaatgtgtgacaaaacaaagttcacatggaagagagctccaacagacagtgggcatgatacagtggtcatggaagtcacattctctggaacaaagccctgtaggatcccagtcagggcagtggcacatggatctccagatgtgaacgtggccatgctgataacgccaaacccaacaattgaaaacaatggaggtggcttcatagagatgcagctgcccccaggggataacatcatctatgttggggaactgagtcatcaatggttccaaaaagggagcagcatcggaagggttttccaaaagaccaagaaaggcatagaaagactgacagtgataggagagcacgcctgggacttcggttctgctggaggctttctgagttcaattgggaaggcggtacatacggtccttggtggcgctttcaacagcatcttcgggggagtggggtttctaccaaaacttttattaggagtggcattggcttggttgggcctgaacatgagaaaccctacaatgtccatgagctttctcttggctggaggtctggtcttggccatgacccttggagtgggggcggatgttggttgcgctgtggacacggaacgaatggagctccgctgtggcgagggcctggtcgtgtggagagaggtctcagaatggtatgacaattatgcctactacccggagacaccgggggcccttgcatcagccataaaggagacatttgaggagggaagctgtggtgtagtcccccagaacaggctcgagatggccatgtggagaagctcggtcacagagctgaatttggctctggcggaaggggaggcaaatctcacagtggtggtggacaagtttgaccccactgactaccgaggtggtgtccctggtttactgaaaaaaggaaaggacataaaagtctcctggaaaagctggggccattcaatgatctggagcattcctgaggccccccgtcgcttcatggtgggcacggaaggacaaagtgagtgtcccctagagagacggaagacaggtgttttcacggtggcagaattcggggttggcctgagaacaaaggtcttcttggatttcagacaggaaccaacacatgagtgtgacacaggagtgatgggagctgcagtcaagaacggcatggcaatccacacagatcaaagtctctggatgagatcaatgaaaaatgacacaggcacttacatagttgaacttttggtcactgacctgaggaactgctcatggcctgctagccacactatcgataatgctgacgtggtggactcagagttattccttccggcgagcctggcaggacccagatcctggtacaacaggatacctggctattcagaacaggtgaaagggccatggaagtacacgcctatccgagttatcagagaggagtgtcccggcacgaccgttaccatcaacgccaagtgtgacaaaagaggagcatctgtgaggagtaccacagagagtggcaaggttatcccagaatggtgctgccgagcgtgcacaatgccaccagtgacgttccggactggaactgattgctggtatgccatggaaatacggccagtccatgaccagggggggcttgttcgctcaatggtggttgcggacaacggtgaattacttagtgagggaggagtccccggaatagtggcattgtttgtggtccttgaatacatcatccgtaggaggccctccacgggaacgacggttgtgtgggggggtatcgtcgttctcgctctgcttgtcaccgggatggtcaggatagagagcctggtgcgctatgtggtggcagtggggatcacattccaccttgagctggggccagagatcgtggccttgatgctactccaggctgtgtttgagctgagggtgggtttgctcagcgcatttgcattgcgcagaagcctcaccgtccgagagatggtgaccacctactttcttttgctggtcctggaattggggctgccgggtgcgagccttgaggagttctggaaatggggtgatgcactggccatgggggcgctgatattcagggcttgcacggcagaaggaaagactggagcggggcttttgctcatggctctcatgacacagcaggatgtggtgactgtgcaccatggactggtgtgcttcctaagtgtagcttcggcatgctcggtctggaggctgctcaagggacacagagagcagaagggattgacctgggttgtccccctggctgggttgcttgggggagagggctctggaatcagactgctggcgttttgggagttgtcagcgcacagaggaagacgatctttcagtgaaccactaactgtggtaggagtcatgctaacactggccagcggcatgatgcgacacacttcccaggaggctctctgtgcactcgcagtggcctcgtttctcttgctgatgctggtgctggggacaagaaagatgcagctggttgccgaatggagtggctgcgttgaatggtatccggaactagtgaatgagggtggagaggttagcctgcgggtccggcaggacgcgatgggtaactttcacttgactgagctcgagaaagaagagagaatgatggctttttggctgattgccggcttggcagcttcggccattcactggtcaggcattcttggtgtgatgggactgtggacgctcacggaaatgctgaggtcatcccgaaggtctgacctggttttctctggacaggggggtcgagagcgtggtgacagacctttcgaggttaaggacggtgtctacaggatttttagccccggcttgttctggggtcagaaccaggtgggagttggctacggttccaagggtgtcttgcacacgatgtggcacgtgacgagaggagcggcgctgtctattgatgacgctgtggccggtccctactgggctgatgtgagggaagatgtcgtgtgttacggaggagcctggagcctggaggaaaaatggaaaggtgaaacagtacaggtccatgccttcccaccggggagggcgcatgaggtgcatcagtgccagcctggggagttgatccttgacaccggaagaaagcttggggcaataccaattgatttggtgaaaggaacatcaggcagccccattctcaacgcccagggagtggttgtggggctatacggaaatggcctaaaaactaatgagacctacgtcagcagcattgctcaaggggaagcggagaagagtcgccccaacctcccacaggctgttgtgggtacgggctggacatcaaagggtcagatcacagtgctggacatgcacccaggctcggggaagacccacagagtcctcccggagctcattcgccaatgcattgacaggcgcctgagaacgttggtgttggctccaactcgtgtggtactcaaagaaatggagcgtgctttgaatgggaaacgggtcaggttccactcaccagcagtcagtgaccaacaggctggaggggcaattgtcgatgtgatgtgtcacgcaacctatgtcaacagaaggctactcccacagggaagacaaaattgggaggtggcaatcatggatgaggcccactggacggacccccacagcatagctgccagaggtcatttgtatactctggcaaaagaaaacaagtgtgcactggtcttgatgacagcgacacctcctggtaagagtgaaccctttccggagtccaatggagccattactagtgaggaaagacagattcctgatggggagtggcgtgacgggtttgactggatcactgagtatgaagggcgcaccgcctggtttgtcccttcgattgcaaaaggtggtgctatagctcgcaccttgagacagaaggggaaaagtgtgatttgtttgaacagcaaaacctttgaaaaggactactccagagtgagggatgagaagcctgactttgtggtgacgactgatatctcggagatgggagctaaccttgacgtgagccgcgtcatagatgggaggacaaacatcaagcccgaggaggttgatgggaaagtcgagctcaccgggaccaggcgagtgaccacggcttccgctgcccaacggcgcggaagagttggtcggcaagacggacgaacagatgaatacatatactctggacagtgtgatgatgatgacagtggattagtgcaatggaaagaggcgcaaatacttcttgacaacataacaaccttgcgggggcccgtggccaccttctatggaccagaacaggacaagatgccggaggtggccggtcactttcgactcactgaagagaaaagaaagcacttccgacatcttctcacccattgtgacttcacaccgtggctggcatggcacgtcgcagcgaatgtatccagcgtcacggatcgaagctggacatgggaagggccggaggcaaatgccgtggatgaggccagtggtgacttggtcacctttaggagcccgaatggggcggagagaactctcaggccggtgtggaaggacgcacgtatgttcaaagagggacgtgacatcaaagagttcgtggcgtacgcgtctgggcgtcgcagcttcggagatgttctgacaggaatgtcgggagttcctgagctcctgcggcacagatgcgtcagtgccctggatgtcttctacacgcttatgcatgaggaacctggcagcagggcaatgagaatggcggagagagatgccccagaggcctttctgactatggttgagatgatggtgctgggtttggcaaccctgggtgtcatctggtgcttcgtcgtccggacttcaatcagccgcatgatgctgggcacgctggtcctgctggcctccttgctactcttgtgggcaggtggcgtcggctatgggaacatggctggagtggctctcatcttttacacgttgctgacggtgctgcagcctgaggcgggaaaacagagaagcagtgacgacaacaaactggcatatttcttgctgacgctctgcagccttgctggactggttgcagccaatgagatgggctttctggagaagaccaaggcagacttgtccacggcgctgtggagtgaacgggaggaaccccggccatggagtgaatggacgaatgtggacatccagccagcgaggtcctgggggacctatgtgctggtggtgtctctgttcacaccttacatcatccaccaactgcagaccaaaatccaacaacttgtcaacagtgccgtggcatctggtgcacaggccatgagagaccttgggggaggtgcccccttctttggtgtggcgggacatgtcatgaccctcggggtggtgtcactgattggggctactcccacctcactgatggtgggcgttggcttggcggcactccatctggccattgtggtgtctggtctggaggctgaattaacacagagagctcataaggtctttttctctgcaatggtgcgcaaccccatggtggatggggatgtcatcaacccattcggggagggggaggcaaaacctgctctatatgaaaggaaaatgagtctggtgttggccacagtgttgtgcctcatgtcggtggtcatgaaccgaacggtggcctccataacagaggcttcagcagtgggactggcagcagcgggacagctgcttagaccggaggctgacacgttgtggacgatgccggttgcttgtggcatgagtggtgtggtcaggggtagcctgtgggggtttttgcctcttgggcatagactctggcttcgagcctctgggggtaggcgtggtggttctgagggagacacgcttggagatctctggaagcggaggctgaacaactgcacgagggaggaattctttgtgtacaggcgcaccggcatcctggagacggaacgtgacaaggctagagagttgctcagaagaggagagaccaatgtgggattggctgtctctcggggcacggcaaagcttgcctggcttgaggaacgcggatatgccaccctcaagggagaggtggtagatcttggatgtggaaggggcggctggtcctattatgcggcatcccgaccggcagtcatgagtgtcagggcatataccattggtggaaaagggcacgaggctccaaagatggtaacaagcctgggttggaacttgattaaattcagatcaggaatggacgtgttcagcatgcagccacaccgggctgacactgtcatgtgtgacatcggagagagcagcccagatgccgctgtggagggtgagaggacaaggaaagtgatactgctcatggagcaatggaaaaacaggaaccccacggctgcctgtgtgttcaaggtgctggccccatatcgcccagaagtgatagaggcactgcacagattccaactgcaatggggggggggtctggtgaggacccctttttcaaggaactccacccatgagatgtattactcaacagccgtcactgggaacatagtgaactccgtcaatgtacagtcgaggaaacttttggctcggtttggagaccagagagggccaaccaaggtgcctgaactcgacctgggagttggaacgaggtgtgtggtcttagctgaggacaaggtgaaagaacaagacgtacaagagaggatcagagcgttgcgggagcaatacagcgaaacctggcatatggacgaggaacacccgtaccggacatggcagtactggggcagctaccgcacggcaccaaccggctcggcggcgtcactgatcaatggggttgtgaaacttctcagctggccatggaacgcacgggaagatgtggtgcgcatggctatgactgacacaacggctttcggacagcagagagtgttcaaagataaagttgacacaaaggcacaggagcctcagcccggtacaagagtcatcatgagagctgtaaatgattggattttggaacgactggcgcagaaaagcaaaccgcgcatgtgcagcagggaagaattcatagcaaaagtgaaatcaaatgcagccttgggagcttggtcagatgagcaaaacagatgggcaagtgcaagagaggctgtagaggatcctgcattctggcgcctcgtggatgaagagagagaaaggcacctcatggggagatgtgcgcactgcgtgtacaacatgatgggcaagagagaaaagaaactgggagagttcggagtggcgaaaggaagtcgggccatttggtacatgtggctggggagtcgctttttggagttcgaggctcttggattcttgaatgaagaccattgggcctctagagagtccagtggagctggagttgagggaataagcttgaactacctgggctggcacctcaagaagttgtcaaccctgaatggaggactcttctatgcagatgacacagctggctgggacacgaaagttaccaatgcagacttagaggatgaagaacagatcctacggtacatggagggtgagcacaaacaattggcaaccacaataatgcaaaaagcataccatgccaaagtcgtgaaggtcgcgaggccttcccgtgatggaggctgcatcatggatgtcatcacaagaagagaccaaagaggttcgggtcaggttgtgacctatgcccttaacaccctcaccaacataaaggtgcaattaatccgaatgatggaaggggaaggggtcatagaggcagcggatgcacacaacccgagactgcttcgagtggagcgctggctgaaagaacacggagaagagcgtcttggaagaatgctcgtcagtggtgacgattgtgtggtgaggcccttggatgacagatttggcaaagcactttactttctgaatgacatggccaagaccaggaaggacattggggaatgggagcactcagccggcttttcaagctgggaggaggtacccttttgttcacaccatttccacgagctagtgatgaaggatggacgcaccctggtggtgccgtgccgagaccaagatgaactcgttgggagggcgcgcatctcaccggggtgcggctggagtgtccgcgagacggcctgcctttcaaaagcctacgggcagatgtggctgctgagctacttccaccgacgagacctgaggacgctcgggcttgccattaactcagcagtgcctgccgattgggttcctaccggccgcacgacgtggagcattcatgccagtggggcctggatgaccacagaagacatgctggacgtttggaaccgggtgtggattctggacaaccctttcatgcagaacaaggaaagggtcatggagtggagggatgttccgtacctccctaaagctcaggacatgttatgttcctcccttgttgggaggagagaaagagcagaatgggccaagaacatctggggagcggtggaaaaggtgaggaagatgataggtcctgaaaagttcaaggactatctctcctgtatggaccgccatgacctgcactgggagctcagactggagagctcaataatctaaacccagaaaaaaaaaaaaaaaaaaaaaaaaaaaaaaaaaaaaaaaaaaaaaaaaaaaaaaaaaaaaaaaaaaaaaaaaaaaaaaaaaaaaaaaaaaaaaaaaaaaaaaaaaaaaaaaaaaaaaaaaaaaaaaaaaaaaaaaaaaaaaaaaaaaaaaccccctgaccagcaaagggggcagaccggtcaggggtgaggaatgcccccagagtgcattacggcagcacgccagtgagagtggcgacgggaaaatggtcgatcccgacgtagggcactctgaaaaattttgtgagaccccctgcatcatgataaggccgaacatggtgcatgaaaggggaggcccccggaagcacgcttccgggaggagggaagagagaaattggcagctctcttcaggatttttcctcctcctatacaaaattccccctcggtagagggggggcggttcttgttctccctgagccaccatcacccagacacaggtagtctgacaaggaggtgatgtgtgactcggaaaaacacccgct